European Patent Specification EP 3 797 174 B1, published July 3, 2024. Title: METHOD AND KIT FOR PREDICTING THE OUTCOME OF AN ASSISTED REPRODUCTIVE TECHNOLOGY PROCEDURE. Applicant: ARTPred BV. The sequence listing filed with the application follows.

SEQUENCE LISTING (2 sequences)

SEQ ID NO: 1 - DNA, 21 bp, Gardnerella vaginalis
ctggatcacctcctttctawg

SEQ ID NO: 2 - DNA, 20 bp, Gardnerella vaginalis
aggcatccrccatgcgccct